European Patent Specification EP 3 501 551 B1, published June 7, 2023. Title: THERAPEUTIC COMPOSITIONS AND METHODS INVOLVING mRNA TRANSFECTION. Applicant: HERZBERG, Mark C. ROSS, Karen F. ZOU, Zianqiong SORENSON, Brent R. Application PCT/US2014/011041. The sequence listing filed with the application follows.

SEQUENCE LISTING (20 sequences)

SEQ ID NO: 1 - skipped

SEQ ID NO: 2 - DNA, 29 bp, artificial
  synthetic oligonucleotide primer
cctaagcttgccaccatggtgagcaaggg

SEQ ID NO: 3 - DNA, 39 bp, artificial
  synthetic oligonucleotide primer
atttgcggccgcttacttgtacagctcgtccatgccgag

SEQ ID NO: 4 - DNA, 37 bp, artificial
  synthetic oligonucleotide primer
cctaagcttgccaccatgaagacccaaagggatggcc

SEQ ID NO: 5 - DNA, 41 bp, artificial
  synthetic oligonucleotide primer
atttgcggccgcctaggactctgtcctgggtacaagattcc

SEQ ID NO: 6 - DNA, 39 bp, artificial
  synthetic oligonucleotide primer
cctaagcttgccaccatgttgaccgagctggagaaagcc

SEQ ID NO: 7 - DNA, 38 bp, artificial
  synthetic oligonucleotide primer
atttgcggccgcctactctttgtggctttcttcatggc

SEQ ID NO: 8 - DNA, 39 bp, artificial
  synthetic oligonucleotide primer
cctaagcttgccaccatgacttgcaaaatgtcgcagctg

SEQ ID NO: 9 - DNA, 30 bp, artificial
  synthetic oligonucleotide primer
atttgcggccgcttagggggtgccctcccc

SEQ ID NO: 10 - DNA, 39 bp, artificial; identical to SEQ ID NO: 6
  synthetic oligonucleotide primer

SEQ ID NO: 11 - DNA, 30 bp, artificial; identical to SEQ ID NO: 9
  synthetic oligonucleotide primer

SEQ ID NO: 12 - skipped

SEQ ID NO: 13 - DNA, 38 bp, artificial
  synthetic oligonucleotide primer
ctagctagcgccaccatgttgaccgagctggagaaagc

SEQ ID NO: 14 - DNA, 35 bp, artificial
  synthetic oligonucleotide primer
ccgctcgagctactctttgtggctttcttcatggc

SEQ ID NO: 15 - DNA, 38 bp, artificial
  synthetic oligonucleotide primer
gctctagagccaccatgacttgcaaaatgtcgcagctg

SEQ ID NO: 16 - DNA, 30 bp, artificial; identical to SEQ ID NO: 9
  synthetic oligonucleotide primer

SEQ ID NO: 17 - DNA, 22 bp, artificial
  synthetic oligonucleotide primer
aaacgtctaggccccccgaacc

SEQ ID NO: 18 - DNA, 34 bp, artificial
  synthetic oligonucleotide primer
tttaacctcgactaaacacatgtaaagcatgtgc

SEQ ID NO: 19 - DNA, 27 bp, artificial
  synthetic oligonucleotide primer
accatgacttgcaaaatgtcgcagctg

SEQ ID NO: 20 - DNA, 31 bp, artificial
  synthetic oligonucleotide primer
attatcatcgtgtttttcaaaggaaaaccac